European Patent Specification EP 3 861 011 B1, published February 11, 2026. Title: BINDERS FOR INHIBITING FORMATION OF MULTIMERIC PROTEINS. Applicant: AFFILOGIC. The sequence listing filed with the application follows.

SEQUENCE LISTING (20 sequences)

SEQ ID NO: 1 - protein, 66 aa, Sulfolobus acidocaldarius
MVKVKFKYKGEEKEVDTSKIKKVWRVGKMVSFTYDDNGKTGRGAVSEKDAPKELLDMLARAEREKK

SEQ ID NO: 2 - protein, 64 aa, Sulfolobus solfataricus
MATVKFKYKGEEKEVDISKIKKVWRVGKMISFTYDEGGGKTGRGAVSEKDAPKELLQMLEKQKK

SEQ ID NO: 3 - protein, 65 aa, Sulfolobus acidocaldarius
MAKVRFKYKGEEKEVDTSKIKKVWRVGKMVSFTYDDNGKTGRGAVSEKDAPKELMDMLARAEKKK

SEQ ID NO: 4 - protein, 64 aa, Sulfolobus shibatae
MVTVKFKYKGEEKEVDTSKIKKVWRVGKMISFTYDEGGGKTGRGAVSEKDAPKELLQMLEKQKK

SEQ ID NO: 5 - protein, 64 aa, Sulfolobus shibatae
MATVKFKYKGEEKQVDISKIKKVWRVGKMISFTYDEGGGKTGRGAVSEKDAPKELLQMLEKQKK

SEQ ID NO: 6 - protein, 64 aa, Sulfolobus tokodaii
MVTVKFKYKGEEKEVDISKIKKVWRVGKMISFTYDDNGKTGRGAVSEKDAPKELLQMLEKSGKK

SEQ ID NO: 7 - protein, 64 aa, Sulfolobus islandicus
MVTVKFKYKGEEKQVDTSKIKKVWRVGKMISFTYDEGGGKTGRGAVSEKDAPKELLQMLEKQKK

SEQ ID NO: 8 - protein, 64 aa, Sulfolobus islandicus
MTTVKFKYKGEEKQVDTSKIKKVWRVGKMISFTYDEGGGKTGRGAVSEKDAPKELLQMLEKQKK

SEQ ID NO: 9 - protein, 64 aa, Sulfolobus islandicus
MTTVKFKYKGEEKQVDISKIKKVWRVGKMISFTYDEGGGKTGRGAVSEKDAPKELLQMLEKQKK

SEQ ID NO: 10 - protein, 62 aa, Metallosphaera sedula.
MATKIKFKYKGQDLEVDISKVKKVWKVGKMVSFTYDDNGKTGRGAVSEKDAPKELLNMIGKK

SEQ ID NO: 11 - protein, 62 aa, Metallosphaera cuprina
MATKIKFKYKGQDLEVDISKVKKVWKVGKMVSFTYDDNGKTGRGAVSEKDAPKELLSMIGKK

SEQ ID NO: 12 - protein, 61 aa, Acidianus hospitalis
MTTVKFKYKGEEKEVDISKIKKVWRVGKMISFTYDDNGKTGRGAVSEKDAPKELLEKLEKK

SEQ ID NO: 13 - protein, 62 aa, Acidianus hospitalis
MATKVKFKYKGEEKEVDISKIKKVWRVGKMISFTYDDNGKTGRGAVSEKDAPKELLDKLEKK

SEQ ID NO: 14 - protein, 60 aa, Acidianus hospitalis
MATKVKFKYKGEEKEVDISKIKKVWRVGKMISFTYDDNGKTGRGAVSEKDAPKELLEKLK

SEQ ID NO: 15 - protein, 68 aa, Artificial Sequence
  Consensus sequence
  VARIANT (2)..(2): Xaa is V, A or T
  VARIANT (3)..(3): Xaa is T or K
  VARIANT (4)..(4): Xaa is - or K
  VARIANT (6)..(6): Xaa is R or K
  VARIANT (15)..(15): Xaa is E or Q
  VARIANT (18)..(18): Xaa is T or I
  VARIANT (31)..(31): Xaa is V or I
  VARIANT (37)..(39): Xaa Xaa Xaa is EGG or DN-
  VARIANT (57)..(57): Xaa is M or L
  VARIANT (58)..(58): Xaa is Q, D or E
  VARIANT (59)..(59): Xaa is M or K
  VARIANT (61)..(67): Xaa is -------, EKS--GK, EK---QK, ARAEREK, ARA-EKK, E-----K, EKS--G, ACAEREK oR ACA-EKK
MXXXVXFKYKGEEKXVDXSKIKKVWRVGKMXSFTYDXXXGKTGRGAVSEKDAPKELXXXLXXXXXXXK

SEQ ID NO: 16 - protein, 65 aa, Artificial Sequence
  Sequence N11 derived from Sac7d
MVKVKFVMFGKEKEVDTSKIVHVMRQGKLVHFWYEDNGKIDKGFVPEKDAPKELLDMLARAEREK

SEQ ID NO: 17 - protein, 65 aa, Artificial Sequence
  Sequence bindig to TNFa derived from N11
  misc_feature (7)..(9): Xaa can be any naturally occurring amino acid
  misc_feature (11)..(11): Xaa can be any naturally occurring amino acid
  misc_feature (21)..(22): Xaa can be any naturally occurring amino acid
  misc_feature (24)..(24): Xaa can be any naturally occurring amino acid
  misc_feature (26)..(26): Xaa can be any naturally occurring amino acid
  misc_feature (29)..(29): Xaa can be any naturally occurring amino acid
  misc_feature (35)..(35): Xaa can be any naturally occurring amino acid
  misc_feature (41)..(41): Xaa can be any naturally occurring amino acid
  misc_feature (44)..(44): Xaa can be any naturally occurring amino acid
  misc_feature (46)..(46): Xaa can be any naturally occurring amino acid
MVKVKFXXXGXEKEVDTSKIXXVXRXGKXVHFWYXDNGKIXKGXVXEKDAPKELLDMLARAEREK

SEQ ID NO: 18 - protein, 65 aa, Artificial Sequence
  Sequence bindig to TNFa derived from N11
  misc_feature (7)..(9): Xaa can be any naturally occurring amino acid
  misc_feature (11)..(11): Xaa can be any naturally occurring amino acid
  misc_feature (21)..(21): Xaa can be any naturally occurring amino acid
  misc_feature (26)..(26): Xaa can be any naturally occurring amino acid
  misc_feature (29)..(29): Xaa can be any naturally occurring amino acid
  misc_feature (35)..(35): Xaa can be any naturally occurring amino acid
  misc_feature (41)..(41): Xaa can be any naturally occurring amino acid
  misc_feature (44)..(44): Xaa can be any naturally occurring amino acid
  misc_feature (46)..(46): Xaa can be any naturally occurring amino acid
MVKVKFXXXGXEKEVDTSKIXHVMRXGKXVHFWYXDNGKIXKGXVXEKDAPKELLDMLARAEREK

SEQ ID NO: 19 - protein, 64 aa, Artificial Sequence
  Sequence F10 derived from Sac7d
VKVKFRSDGEEKEVDTSKILLVARQGKIVMFGYDDNGKPGIGLVWEKDDPKELLDMLARAERGK

SEQ ID NO: 20 - protein, 64 aa, Artificial Sequence
  Sequence derived from F10
VKVKFRSDGEEKEVDTSKILLVARQGKIVMFGYDDNGKPGIGLVWEKDDPKELLDMLARAEREK